European Patent Application EP 4 397 750 A1, published July 10, 2024. Title: Methods for producing inner ear stria vascularis marginal cells, methods for evaluating drugs, and cell cultures for drug evaluation. Applicant: The Kitasato Institute. Application JP. The sequence listing filed with the application follows.

SEQUENCE LISTING (8 sequences)

SEQ ID NO: 1 - DNA, 23 bp, human
  source 1..23: mol_type = other DNA
tcaagtcgagtctatctgcatcc

SEQ ID NO: 2 - DNA, 21 bp, human
  source 1..21: mol_type = other DNA
catgtcacgaccagtcacaac

SEQ ID NO: 3 - DNA, 20 bp, human
  source 1..20: mol_type = other DNA
gcccagtgtcagctccatta

SEQ ID NO: 4 - DNA, 21 bp, human
  source 1..21: mol_type = other DNA
gctgtccatagggaggttgaa

SEQ ID NO: 5 - DNA, 23 bp, human
  source 1..23: mol_type = other DNA
caaagtgagacctgccaaaaaga

SEQ ID NO: 6 - DNA, 21 bp, human
  source 1..21: mol_type = other DNA
tggacaagggatctgacagtg

SEQ ID NO: 7 - DNA, 20 bp, human
  source 1..20: mol_type = other DNA
tgaagtgtgacgtggacatc

SEQ ID NO: 8 - DNA, 20 bp, human
  source 1..20: mol_type = other DNA
ggaggagcaatgatcttgat